European Patent Application EP 4 497 435 A1, published January 29, 2025. Title: Skeletal muscle potentiator. Applicant: Sato Pharmaceutical Co., Ltd. The sequence listing filed with the application follows.

SEQUENCE LISTING (6 sequences)

SEQ ID NO: 1 - DNA, 19 bp, synthetic construct
  misc_feature 1..19: note = Trim63 sense primer
  source 1..19: mol_type = other DNA
ccaggctgcgaatccctac

SEQ ID NO: 2 - DNA, 23 bp, synthetic construct
  misc_feature 1..23: note = Trim63 antisense primer
  source 1..23: mol_type = other DNA
attttctcgtcttcgtgttcctt

SEQ ID NO: 3 - DNA, 22 bp, synthetic construct
  misc_feature 1..22: note = Mstn sense primer
  source 1..22: mol_type = other DNA
agtggatctaaatgagggcagt

SEQ ID NO: 4 - DNA, 19 bp, synthetic construct
  misc_feature 1..19: note = Mstn antisense primer
  source 1..19: mol_type = other DNA
gtttccaggcgcagcttac

SEQ ID NO: 5 - DNA, 24 bp, synthetic construct
  misc_feature 1..24: note = Gapdh sense primer
  source 1..24: mol_type = other DNA
tcaacagcaactcccactcttcca

SEQ ID NO: 6 - DNA, 24 bp, synthetic construct
  misc_feature 1..24: note = Gapdh antisense primer
  source 1..24: mol_type = other DNA
accctgttgctgtagccgtattca